European Patent Specification EP 3 733 196 B1, published August 30, 2023. Title: PHARMACEUTICAL COMPOSITION COMPRISING PEPTIDO TYPE APL. Applicant: CENTER OF GENETIC ENGINEERING AND BIOTECHNOLOGY. Application CU 2017-0176. The sequence listing filed with the application follows.

SEQUENCE LISTING (1 sequence)

SEQ ID NO: 1 - protein, 27 aa, Artificial Sequence
  Description of the Artificial Sequence: Peptide APL type
SIDLKDKYKNIGAKLVQLVANNTNEEA